European Patent Application EP 4 538 284 A1, published April 16, 2025. Title: Novel Engineered Streptolysin O Derived Epitopes. Applicant: Tanea Medical AB. The sequence listing filed with the application follows.

SEQUENCE LISTING (12 sequences)

SEQ ID NO: 1 - protein, 571 aa, Streptococcus pyogenes
MSNKKTFKKYSRVAGLLTAALIIGNLVTANAESNKQNTASTETTTTNEQPKPESSELTTEKAGQKTDDMLNSNDMIKLAPKEMPLESAEKEEKKSEDKKKSEEDHTEEINDKIYSLNYNELEVLAKNGETIENFVPKEGVKKADKFIVIERKKKNINTTPVDISIIDSVTDRTYPAALQLANKGFTENKPDAVVTKRNPQKIHIDLPGMGDKATVEVNDPTYANVSTAIDNLVNQWHDNYSGGNTLPARTQYTESMVYSKSQIEAALNVNSKILDGTLGIDFKSISKGEKKVMIAAYKQIFYTVSANLPNNPADVFDKSVTFKELQRKGVSNEAPPLFVSNVAYGRTVFVKLETSSKSNDVEAAFSAALKGTDVKTNGKYSDILENSSFTAVVLGGDAAEHNKVVTKDFDVIRNVIKDNATFSRKNPAYPISYTSVFLKNNKIAGVNNRTEYVETTSTEYTSGKINLSHQGAYVAQYEILWDEINYDDKGKEVITKRRWDNNWYSKTSPFSTVIPLGANSRNIRIMARECTGLAWEWWRKVIDERDVKLSKEINVNISGSTLSPYGSITYK

SEQ ID NO: 2 - protein, 171 aa, Streptococcus pyogenes
TQYTESMVYSKSQIEAALNVNSKILDGTLGIDFKSISKGEKKVMIAAYKQIFYTVSANLPNNPADVFDKSVTFKELQRKGVSNEAPPLFVSNVAYGRTVFVKLETSSKSNDVEAAFSAALKGTDVKTNGKYSDILENSSFTAVVLGGDAAEHNKVVTKDFDVIRNVIKDNA

SEQ ID NO: 3 - protein, 49 aa, Streptococcus pyogenes
TQYTESMVYSKSQIEAALNVNSKILDGTLGIDFKSISKGEKKVMIAAYK

SEQ ID NO: 4 - protein, 47 aa, Streptococcus pyogenes
QIFYTVSANLPNNPADVFDKSVTFKELQRKGVSNEAPPLFVSNVAYG

SEQ ID NO: 5 - protein, 75 aa, Streptococcus pyogenes
RTVFVKLETSSKSNDVEAAFSAALKGTDVKTNGKYSDILENSSFTAVVLGGDAAEHNKVVTKDFDVIRNVIKDNA

SEQ ID NO: 6 - protein, 128 aa, Synthetic construct
TQYTESMVYSKSQIEAALNVNSKILDGTLGIDFKSISKGEKKVMIAAYKAPNGRTVFVKLETSSKSNDVEAAFSAALKGTDVKTNGKYSDILENSSFTAVVLGGDAAEHNKVVTKDFDVIRNVIKDNA

SEQ ID NO: 7 - protein, 128 aa, Synthetic construct
TQYTESMVYSKSQIEAALNVNSKILDGTLGIDFKSISKGEKKVMIAAYKAPGGRTVFVKLETSSKSNDVEAAFSAALKGTDVKTNGKYSDILENSSFTAVVLGGDAAEHNKVVTKDFDVIRNVIKDNA

SEQ ID NO: 8 - protein, 128 aa, Synthetic construct
TQYTESMVYSKSQIEAALNVNSKILDGTLGIDFKSISKGEKKVMIAAYKCPNGRTVFVKLETSSKSNDVEAAFSAALKGTDVKTNGKYSDILENSSFTAVVLGGDAAEHNKVVTKDFDVIRNVIKDNA

SEQ ID NO: 9 - protein, 128 aa, Synthetic construct
TQYTESMVYSKSQIEAALNVNSKILDGTLGIDFKSISKGEKKVMIAAYKCPGGRTVFVKLETSSKSNDVEAAFSAALKGTDVKTNGKYSDILENSSFTAVVLGGDAAEHNKVVTKDFDVIRNVIKDNA

SEQ ID NO: 10 - protein, 119 aa, Synthetic construct
EEAELAYLLGELAYKLGEYRIAIRAYRIALKRDPNNAEAWYNLGNAYYKQGRYREAIEYYQKALELDPNNAEAWYNLGNAYYERGEYEEAIEYYRKALRLDPNNADAMQNLLNAKMREE

SEQ ID NO: 11 - protein, 10 aa, Synthetic construct
WELQHHHHHH

SEQ ID NO: 12 - protein, 6 aa, Synthetic construct
HHHHHH